European Patent Specification EP 3 366 693 B1, published August 16, 2023. Title: Cyclic peptides. Applicant: Fuji Film Corporation. The sequence listing filed with the application follows.

SEQUENCE LISTING (91 sequences)

SEQ ID NO: 1 - protein, 9 aa, Artificial Sequence
  Sequence-1
AYHLGELVW

SEQ ID NO: 2 - protein, 9 aa, Artificial Sequence
  Sequence-2
AYHRGELVW

SEQ ID NO: 3 - protein, 15 aa, Artificial Sequence
  Cyclic_peptide_1
  MISC_FEATURE (2)..(2): Xaa2 is an amino acid residue derived from N-epsilon-chloroacetyl-L-lysine. Xaa12 is an amino acid residue derived from L-homocysteine. Xaa2 and Xaa12 are bridged by a thioether bond.
  MISC_FEATURE (12)..(12): Xaa2 is an amino acid residue derived from N-epsilon-chloroacetyl-L-lysine. Xaa12 is an amino acid residue derived from L-homocysteine. Xaa2 and Xaa12 are bridged by a thioether bond.
DXAYHRGELVWXTKK

SEQ ID NO: 4 - protein, 15 aa, Artificial Sequence
  Cyclic_peptide_2
  MISC_FEATURE (2)..(2): Xaa2 and Xaa12 are amino acid residues derived from L-homocysteine. Xaa2 and Xaa12 are bridged by a disulfide bond.
  MISC_FEATURE (12)..(12): Xaa2 and Xaa12 are amino acid residues derived from L-homocysteine. Xaa2 and Xaa12 are bridged by a disulfide bond.
DXAYHRGELVWXTKK

SEQ ID NO: 5 - protein, 15 aa, Artificial Sequence
  Cyclic_peptide_3
  MISC_FEATURE (2)..(2): Xaa2 is an amino acid residue derived from L-homocysteine. Xaa12 is an amino acid residue derived from N-delta-chloroacetyl-L-ornithine. Xaa2 and Xaa12 are bridged by a thioether bond.
  MISC_FEATURE (12)..(12): Xaa2 is an amino acid residue derived from L-homocysteine. Xaa12 is an amino acid residue derived from N-delta-chloroacetyl-L-ornithine. Xaa2 and Xaa12 are bridged by a thioether bond.
DXAYHRGELVWXTKK

SEQ ID NO: 6 - protein, 15 aa, Artificial Sequence
  Cyclic_peptide_4
  MISC_FEATURE (4)..(4): Xaa4 is an amino acid residue derived from N-epsilon-cloroacetyl-L-lysine. Xaa14 is an amino acid residue derived from L-homocysteine. Xaa4 and Xaa14 are bridged by a thioether bond.
  MISC_FEATURE (14)..(14): Xaa4 is an amino acid residue derived from N-epsilon-cloroacetyl-L-lysine. Xaa14 is an amino acid residue derived from L-homocysteine. Xaa4 and Xaa14 are bridged by a thioether bond.
KKDXAYHRGELVWXT

SEQ ID NO: 7 - protein, 15 aa, Artificial Sequence
  Cyclic_peptide_5
  MISC_FEATURE (2)..(2): Xaa2 is an amino acid residue derived from N-epsilon-chloroacetyl-L-lysine. Xaa12 is an amino acid residue derived from L-homocysteine. Xaa2 and Xaa12 are bridged by a thioether bond.
  MISC_FEATURE (12)..(12): Xaa2 is an amino acid residue derived from N-epsilon-chloroacetyl-L-lysine. Xaa12 is an amino acid residue derived from L-homocysteine. Xaa2 and Xaa12 are bridged by a thioether bond.
DXAYHLGELVWXTKK

SEQ ID NO: 8 - protein, 15 aa, Artificial Sequence
  Cyclic_peptide_6
  MISC_FEATURE (2)..(2): Xaa2 and Xaa12 are amino acid residues derived from L-homocysteine. Xaa2 and Xaa12 are bridged by a disulfide bond.
  MISC_FEATURE (12)..(12): Xaa2 and Xaa12 are amino acid residues derived from L-homocysteine. Xaa2 and Xaa12 are bridged by a disulfide bond.
DXAYHLGELVWXTKK

SEQ ID NO: 9 - protein, 15 aa, Artificial Sequence
  Cyclic_peptide_7
  MISC_FEATURE (2)..(2): Xaa2 is an amino acid residue derived from (2S)-2-amino-3-[(2-chloroacetyl)amino]propanoic acid. Xaa12 is an amino acid residue derived from L-homocysteine. Xaa2 and Xaa12 are bridged by a thioether bond.
  MISC_FEATURE (12)..(12): Xaa2 is an amino acid residue derived from (2S)-2-amino-3-[(2-chloroacetyl)amino]propanoic acid. Xaa12 is an amino acid residue derived from L-homocysteine. Xaa2 and Xaa12 are bridged by a thioether bond.
DXAYHLGELVWXTKK

SEQ ID NO: 10 - protein, 15 aa, Artificial Sequence
  Cyclic_peptide_8
  MISC_FEATURE (2)..(2): Xaa2 is an amino acid residue derived from (2S)-2amino-4-[(2-chloroacetyl)amino]butanoic acid. Xaa12 is an amino acid residue derived from L-homocysteine. Xaa2 and Xaa12 are bridged by a thioether bond.
  MISC_FEATURE (12)..(12): Xaa2 is an amino acid residue derived from (2S)-2amino-4-[(2-chloroacetyl)amino]butanoic acid. Xaa12 is an amino acid residue derived from L-homocysteine. Xaa2 and Xaa12 are bridged by a thioether bond.
DXAYHLGELVWXTKK

SEQ ID NO: 11 - protein, 15 aa, Artificial Sequence
  Cyclic_peptide_9
  MISC_FEATURE (2)..(2): Xaa2 is an amino acid residue derived from N-delta-chloroacetyl-L-ornithine. Xaa12 is an amino acid residue derived from L-homocysteine. Xaa2 and Xaa12 are bridged by a thioether bond.
  MISC_FEATURE (12)..(2): Xaa2 is an amino acid residue derived from N-delta-chloroacetyl-L-ornithine. Xaa12 is an amino acid residue derived from L-homocysteine. Xaa2 and Xaa12 are bridged by a thioether bond.
  misc_feature (12)..(12): Xaa can be any naturally occurring amino acid
DXAYHLGELVWXTKK

SEQ ID NO: 12 - protein, 15 aa, Artificial Sequence
  Cyclic_peptide_10
  MISC_FEATURE (2)..(2): Xaa2 is an amino acid residue derived from L-homocysteine. Xaa12 is an amino acid residue derived from (2S)-2-amino-4-[(2-chloroacetyl)amino]butanoic acid. Xaa2 and Xaa12 are bridged by a thioether bond.
  MISC_FEATURE (12)..(12): Xaa2 is an amino acid residue derived from L-homocysteine. Xaa12 is an amino acid residue derived from (2S)-2-amino-4-[(2-chloroacetyl)amino]butanoic acid. Xaa2 and Xaa12 are bridged by a thioether bond.
DXAYHLGELVWXTKK

SEQ ID NO: 13 - protein, 15 aa, Artificial Sequence
  Cyclic_peptide_11
  MISC_FEATURE (2)..(2): Xaa2 is an amino acid residue derived from homocysteine. Xaa12 is an amino acid residue derived from N-delta-chloroacetyl-L-ornithine. Xaa2 and Xaa12 are bridged by a thioether bond.
  MISC_FEATURE (12)..(12): Xaa2 is an amino acid residue derived from homocysteine. Xaa12 is an amino acid residue derived from N-delta-chloroacetyl-L-ornithine. Xaa2 and Xaa12 are bridged by a thioether bond.
DXAYHLGELVWXTKK

SEQ ID NO: 14 - protein, 15 aa, Artificial Sequence
  Cyclic_peptide_12
  MISC_FEATURE (2)..(2): Xaa2 is an amino acid residue derived from L-homocysteine. Xaa12 is an amino acid residue derived from N-epsilon-chloroacetyl-L-lysine. Xaa2 and Xaa12 are bridged by a thioether bond.
  MISC_FEATURE (12)..(12): Xaa2 is an amino acid residue derived from L-homocysteine. Xaa12 is an amino acid residue derived from N-epsilon-chloroacetyl-L-lysine. Xaa2 and Xaa12 are bridged by a thioether bond.
DXAYHLGELVWXTKK

SEQ ID NO: 15 - protein, 15 aa, Artificial Sequence
  Cyclic_peptide_13
  MISC_FEATURE (2)..(2): Xaa2 is an amino acid residue derived from N-epsilon-chloroacetyl-L-lysine. Xaa12 is an amino acid residue derived from L-homocysteine. Xaa2 and Xaa12 are bridged by a thioether bond.
  MISC_FEATURE (12)..(12): Xaa2 is an amino acid residue derived from N-epsilon-chloroacetyl-L-lysine. Xaa12 is an amino acid residue derived from L-homocysteine. Xaa2 and Xaa12 are bridged by a thioether bond.
DXAYHLGELVWXSKK

SEQ ID NO: 16 - protein, 15 aa, Artificial Sequence
  Cyclic_peptide_14
  MISC_FEATURE (2)..(2): Xaa2 is an amino acid residue derived from N-epsilon-chloroacetyl-L-lysine. Xaa12 is an amino acid residue derived from L-homocysteine. Xaa2 and Xaa12 are bridged by a thioether bond.
  MISC_FEATURE (12)..(12): Xaa2 is an amino acid residue derived from N-epsilon-chloroacetyl-L-lysine. Xaa12 is an amino acid residue derived from L-homocysteine. Xaa2 and Xaa12 are bridged by a thioether bond.
  MISC_FEATURE (13)..(13): Xaa13 is an amino acid residue derived from L-homoserine.
DXAYHLGELVWXXKK

SEQ ID NO: 17 - protein, 15 aa, Artificial Sequence
  Cyclic_peptide_15
  MISC_FEATURE (2)..(2): Xaa2 is an amino acid residue derived from N-epsilon-chloroacetyl-L-lysine. Xaa12 is an amino acid residue derived from L-homocysteine. Xaa2 and Xaa12 are bridged by a thioether bond.
  MISC_FEATURE (12)..(12): Xaa2 is an amino acid residue derived from N-epsilon-chloroacetyl-L-lysine. Xaa12 is an amino acid residue derived from L-homocysteine. Xaa2 and Xaa12 are bridged by a thioether bond.
DXAYHLGELVWXDKK

SEQ ID NO: 18 - protein, 15 aa, Artificial Sequence
  Cyclic_peptide_16
  MISC_FEATURE (2)..(2): Xaa2 is an amino acid residue derived from N-epsilon-chloroacetyl-L-lysine. Xaa12 is an amino acid residue derived from L-homocysteine. Xaa2 and Xaa12 are bridged by a thioether bond.
  MISC_FEATURE (12)..(12): Xaa2 is an amino acid residue derived from N-epsilon-chloroacetyl-L-lysine. Xaa12 is an amino acid residue derived from L-homocysteine. Xaa2 and Xaa12 are bridged by a thioether bond.
DXAYHLGELVWXEKK

SEQ ID NO: 19 - protein, 15 aa, Artificial Sequence
  Cyclic_peptide_17
  MISC_FEATURE (2)..(2): Xaa2 is an amino acid residue derived from N-epsilon-chloroacetyl-L-lysine. Xaa12 is an amino acid residue derived from L-homocysteine. Xaa2 and Xaa12 are bridged by a thioether bond.
  MISC_FEATURE (12)..(12): Xaa2 is an amino acid residue derived from N-epsilon-chloroacetyl-L-lysine. Xaa12 is an amino acid residue derived from L-homocysteine. Xaa2 and Xaa12 are bridged by a thioether bond.
DXAYHLGELVWXYKK

SEQ ID NO: 20 - protein, 15 aa, Artificial Sequence
  Cyclic_peptide_18
  MISC_FEATURE (2)..(2): Xaa2 is an amino acid residue derived from N-epsilon-chloroacetyl-L-lysine. Xaa12 is an amino acid residue derived from L-homocysteine. Xaa2 and Xaa12 are bridged by a thioether bond.
  MISC_FEATURE (12)..(12): Xaa2 is an amino acid residue derived from N-epsilon-chloroacetyl-L-lysine. Xaa12 is an amino acid residue derived from L-homocysteine. Xaa2 and Xaa12 are bridged by a thioether bond.
  MISC_FEATURE (13)..(13): Xaa13 is an amino acid residue derived from L-homotyrosine.
DXAYHLGELVWXXKK

SEQ ID NO: 21 - protein, 15 aa, Artificial Sequence
  Cyclic_peptide_19
  MISC_FEATURE (2)..(2): Xaa2 is an amino acid residue derived from N-epsilon-chloroacetyl-L-lysine. Xaa12 is an amino acid residue derived from L-homocysteine. Xaa2 and Xaa12 are bridged by a thioether bond.
  MISC_FEATURE (12)..(12): Xaa2 is an amino acid residue derived from N-epsilon-chloroacetyl-L-lysine. Xaa12 is an amino acid residue derived from L-homocysteine. Xaa2 and Xaa12 are bridged by a thioether bond.
SXAYHLGELVWXTKK

SEQ ID NO: 22 - protein, 15 aa, Artificial Sequence
  Cyclic_peptide_20
  MISC_FEATURE (2)..(2): Xaa2 is an amino acid residue derived from N-epsilon-chloroacetyl-L-lysine. Xaa12 is an amino acid residue derived from L-homocysteine. Xaa2 and Xaa12 are bridged by a thioether bond.
  MISC_FEATURE (12)..(12): Xaa2 is an amino acid residue derived from N-epsilon-chloroacetyl-L-lysine. Xaa12 is an amino acid residue derived from L-homocysteine. Xaa2 and Xaa12 are bridged by a thioether bond.
TXAYHLGELVWXTKK

SEQ ID NO: 23 - protein, 15 aa, Artificial Sequence
  Cyclic_peptide_21
  MISC_FEATURE (1)..(1): Xaa1 is an amino acid residue derived from L-homoserine.
  MISC_FEATURE (2)..(2): Xaa2 is an amino acid residue derived from N-epsilon-chloroacetyl-L-lysine. Xaa12 is an amino acid residue derived from L-homocysteine. Xaa2 and Xaa12 are bridged by a thioether bond.
  MISC_FEATURE (12)..(12): Xaa2 is an amino acid residue derived from N-epsilon-chloroacetyl-L-lysine. Xaa12 is an amino acid residue derived from L-homocysteine. Xaa2 and Xaa12 are bridged by a thioether bond.
XXAYHLGELVWXTKK

SEQ ID NO: 24 - protein, 15 aa, Artificial Sequence
  Cyclic_peptide_22
  MISC_FEATURE (2)..(2): Xaa2 is an amino acid residue derived from N-epsilon-chloroacetyl-L-lysine. Xaa12 is an amino acid residue derived from L-homocysteine. Xaa2 and Xaa12 are bridged by a thioether bond.
  MISC_FEATURE (12)..(12): Xaa2 is an amino acid residue derived from N-epsilon-chloroacetyl-L-lysine. Xaa12 is an amino acid residue derived from L-homocysteine. Xaa2 and Xaa12 are bridged by a thioether bond.
EXAYHLGELVWXTKK

SEQ ID NO: 25 - protein, 16 aa, Artificial Sequence
  Cyclic_peptide_23
  MISC_FEATURE (2)..(2): Xaa2 is an amino acid residue derived from N-epsilon-chloroacetyl-L-lysine. Xaa12 is an amino acid residue derived from L-homocysteine. Xaa2 and Xaa12 are bridged by a thioether bond.
  MISC_FEATURE (12)..(12): Xaa2 is an amino acid residue derived from N-epsilon-chloroacetyl-L-lysine. Xaa12 is an amino acid residue derived from L-homocysteine. Xaa2 and Xaa12 are bridged by a thioether bond.
  misc_feature (13)..(13): Xaa can be any naturally occurring amino acid
DXAAYHLGELVWXTKK

SEQ ID NO: 26 - protein, 17 aa, Artificial Sequence
  Cyclic_peptide_24
  MISC_FEATURE (2)..(2): Xaa2 is an amino acid residue derived from N-epsilon-chloroacetyl-L-lysine. Xaa12 is an amino acid residue derived from L-homocysteine. Xaa2 and Xaa12 are bridged by a thioether bond.
  MISC_FEATURE (12)..(12): Xaa2 is an amino acid residue derived from N-epsilon-chloroacetyl-L-lysine. Xaa12 is an amino acid residue derived from L-homocysteine. Xaa2 and Xaa12 are bridged by a thioether bond.
  misc_feature (14)..(14): Xaa can be any naturally occurring amino acid
DXAAAYHLGELVWXTKK

SEQ ID NO: 27 - protein, 18 aa, Artificial Sequence
  Cyclic_peptide_25
  MISC_FEATURE (2)..(2): Xaa2 is an amino acid residue derived from N-epsilon-chloroacetyl-L-lysine. Xaa12 is an amino acid residue derived from L-homocysteine. Xaa2 and Xaa12 are bridged by a thioether bond.
  MISC_FEATURE (12)..(12): Xaa2 is an amino acid residue derived from N-epsilon-chloroacetyl-L-lysine. Xaa12 is an amino acid residue derived from L-homocysteine. Xaa2 and Xaa12 are bridged by a thioether bond.
  misc_feature (15)..(15): Xaa can be any naturally occurring amino acid
DXAAAAYHLGELVWXTKK

SEQ ID NO: 28 - protein, 15 aa, Artificial Sequence
  Cyclic_peptide_26
  MISC_FEATURE (2)..(2): Xaa2 is an amino acid residue derived from N-epsilon-chloroacetyl-L-lysine. Xaa12 is an amino acid residue derived from L-homocysteine. Xaa2 and Xaa12 are bridged by a thioether bond.
  MISC_FEATURE (12)..(12): Xaa2 is an amino acid residue derived from N-epsilon-chloroacetyl-L-lysine. Xaa12 is an amino acid residue derived from L-homocysteine. Xaa2 and Xaa12 are bridged by a thioether bond.
DXSYHLGELVWXTKK

SEQ ID NO: 29 - protein, 15 aa, Artificial Sequence
  Cyclic_peptide_27
  MISC_FEATURE (2)..(2): Xaa2 is an amino acid residue derived from N-epsilon-chloroacetyl-L-lysine. Xaa12 is an amino acid residue derived from L-homocysteine. Xaa2 and Xaa12 are bridged by a thioether bond.
  MISC_FEATURE (12)..(12): Xaa2 is an amino acid residue derived from N-epsilon-chloroacetyl-L-lysine. Xaa12 is an amino acid residue derived from L-homocysteine. Xaa2 and Xaa12 are bridged by a thioether bond.
DXTYHLGELVWXTKK

SEQ ID NO: 30 - protein, 15 aa, Artificial Sequence
  Cyclic_peptide_28
  MISC_FEATURE (2)..(2): Xaa2 is an amino acid residue derived from N-epsilon-chloroacetyl-L-lysine. Xaa12 is an amino acid residue derived from L-homocysteine. Xaa2 and Xaa12 are bridged by a thioether bond.
  MISC_FEATURE (12)..(12): Xaa2 is an amino acid residue derived from N-epsilon-chloroacetyl-L-lysine. Xaa12 is an amino acid residue derived from L-homocysteine. Xaa2 and Xaa12 are bridged by a thioether bond.
DXAFHLGELVWXTKK

SEQ ID NO: 31 - protein, 15 aa, Artificial Sequence
  Cyclic_peptide_29
  MISC_FEATURE (2)..(2): Xaa2 is an amino acid residue derived from N-epsilon-chloroacetyl-L-lysine. Xaa12 is an amino acid residue derived from L-homocysteine. Xaa2 and Xaa12 are bridged by a thioether bond.
  MISC_FEATURE (12)..(12): Xaa2 is an amino acid residue derived from N-epsilon-chloroacetyl-L-lysine. Xaa12 is an amino acid residue derived from L-homocysteine. Xaa2 and Xaa12 are bridged by a thioether bond.
DXAHHLGELVWXTKK

SEQ ID NO: 32 - protein, 15 aa, Artificial Sequence
  Cyclic_peptide_30
  MISC_FEATURE (2)..(2): Xaa2 is an amino acid residue derived from N-epsilon-chloroacetyl-L-lysine. Xaa12 is an amino acid residue derived from L-homocysteine. Xaa2 and Xaa12 are bridged by a thioether bond.
  MISC_FEATURE (12)..(12): Xaa2 is an amino acid residue derived from N-epsilon-chloroacetyl-L-lysine. Xaa12 is an amino acid residue derived from L-homocysteine. Xaa2 and Xaa12 are bridged by a thioether bond.
DXAVHLGELVWXTKK

SEQ ID NO: 33 - protein, 15 aa, Artificial Sequence
  Cyclic_peptide_31
  MISC_FEATURE (2)..(2): Xaa2 is an amino acid residue derived from N-epsilon-chloroacetyl-L-lysine. Xaa12 is an amino acid residue derived from L-homocysteine. Xaa2 and Xaa12 are bridged by a thioether bond.
  MISC_FEATURE (12)..(12): Xaa2 is an amino acid residue derived from N-epsilon-chloroacetyl-L-lysine. Xaa12 is an amino acid residue derived from L-homocysteine. Xaa2 and Xaa12 are bridged by a thioether bond.
DXAMHLGELVWXTKK

SEQ ID NO: 34 - protein, 15 aa, Artificial Sequence
  Cyclic_peptide_32
  MISC_FEATURE (2)..(2): Xaa2 is an amino acid residue derived from N-epsilon-chloroacetyl-L-lysine. Xaa12 is an amino acid residue derived from L-homocysteine. Xaa2 and Xaa12 are bridged by a thioether bond.
  MISC_FEATURE (12)..(12): Xaa2 is an amino acid residue derived from N-epsilon-chloroacetyl-L-lysine. Xaa12 is an amino acid residue derived from L-homocysteine. Xaa2 and Xaa12 are bridged by a thioether bond.
DXAYYLGELVWXTKK

SEQ ID NO: 35 - protein, 15 aa, Artificial Sequence
  Cyclic_peptide_33
  MISC_FEATURE (2)..(2): Xaa2 is an amino acid residue derived from N-epsilon-chloroacetyl-L-lysine. Xaa12 is an amino acid residue derived from L-homocysteine. Xaa2 and Xaa12 are bridged by a thioether bond.
  MISC_FEATURE (12)..(12): Xaa2 is an amino acid residue derived from N-epsilon-chloroacetyl-L-lysine. Xaa12 is an amino acid residue derived from L-homocysteine. Xaa2 and Xaa12 are bridged by a thioether bond.
DXAYWLGELVWXTKK

SEQ ID NO: 36 - protein, 15 aa, Artificial Sequence
  Cyclic_peptide_34
  MISC_FEATURE (2)..(2): Xaa2 is an amino acid residue derived from N-epsilon-chloroacetyl-L-lysine. Xaa12 is an amino acid residue derived from L-homocysteine. Xaa2 and Xaa12 are bridged by a thioether bond.
  MISC_FEATURE (12)..(12): Xaa2 is an amino acid residue derived from N-epsilon-chloroacetyl-L-lysine. Xaa12 is an amino acid residue derived from L-homocysteine. Xaa2 and Xaa12 are bridged by a thioether bond.
DXAYHMGELVWXTKK

SEQ ID NO: 37 - protein, 15 aa, Artificial Sequence
  Cyclic_peptide_35
  MISC_FEATURE (2)..(2): Xaa2 is an amino acid residue derived from N-epsilon-chloroacetyl-L-lysine. Xaa12 is an amino acid residue derived from L-homocysteine. Xaa2 and Xaa12 are bridged by a thioether bond.
  MISC_FEATURE (12)..(12): Xaa2 is an amino acid residue derived from N-epsilon-chloroacetyl-L-lysine. Xaa12 is an amino acid residue derived from L-homocysteine. Xaa2 and Xaa12 are bridged by a thioether bond.
DXAYHFGELVWXTKK

SEQ ID NO: 38 - protein, 15 aa, Artificial Sequence
  Cyclic_peptide_36
  MISC_FEATURE (2)..(2): Xaa2 is an amino acid residue derived from N-epsilon-chloroacetyl-L-lysine. Xaa12 is an amino acid residue derived from L-homocysteine. Xaa2 and Xaa12 are bridged by a thioether bond.
  MISC_FEATURE (12)..(12): Xaa2 is an amino acid residue derived from N-epsilon-chloroacetyl-L-lysine. Xaa12 is an amino acid residue derived from L-homocysteine. Xaa2 and Xaa12 are bridged by a thioether bond.
DXAYHHGELVWXTKK

SEQ ID NO: 39 - protein, 15 aa, Artificial Sequence
  Cyclic_peptide_37
  MISC_FEATURE (2)..(2): Xaa2 is an amino acid residue derived from N-epsilon-chloroacetyl-L-lysine. Xaa12 is an amino acid residue derived from L-homocysteine. Xaa2 and Xaa12 are bridged by a thioether bond.
  MISC_FEATURE (12)..(12): Xaa2 is an amino acid residue derived from N-epsilon-chloroacetyl-L-lysine. Xaa12 is an amino acid residue derived from L-homocysteine. Xaa2 and Xaa12 are bridged by a thioether bond.
DXAYHVGELVWXTKK

SEQ ID NO: 40 - protein, 15 aa, Artificial Sequence
  Cyclic_peptide_38
  MISC_FEATURE (2)..(2): Xaa2 is an amino acid residue derived from N-epsilon-chloroacetyl-L-lysine. Xaa12 is an amino acid residue derived from L-homocysteine. Xaa2 and Xaa12 are bridged by a thioether bond.
  MISC_FEATURE (12)..(12): Xaa2 is an amino acid residue derived from N-epsilon-chloroacetyl-L-lysine. Xaa12 is an amino acid residue derived from L-homocysteine. Xaa2 and Xaa12 are bridged by a thioether bond.
DXAYHIGELVWXTKK

SEQ ID NO: 41 - protein, 15 aa, Artificial Sequence
  Cyclic_peptide_39
  MISC_FEATURE (2)..(2): Xaa2 is an amino acid residue derived from N-epsilon-chloroacetyl-L-lysine. Xaa12 is an amino acid residue derived from L-homocysteine. Xaa2 and Xaa12 are bridged by a thioether bond.
  MISC_FEATURE (12)..(12): Xaa2 is an amino acid residue derived from N-epsilon-chloroacetyl-L-lysine. Xaa12 is an amino acid residue derived from L-homocysteine. Xaa2 and Xaa12 are bridged by a thioether bond.
DXAYHNGELVWXTKK

SEQ ID NO: 42 - protein, 15 aa, Artificial Sequence
  Cyclic_peptide_40
  MISC_FEATURE (2)..(2): Xaa2 is an amino acid residue derived from N-epsilon-chloroacetyl-L-lysine. Xaa12 is an amino acid residue derived from L-homocysteine. Xaa2 and Xaa12 are bridged by a thioether bond.
  MISC_FEATURE (12)..(12): Xaa2 is an amino acid residue derived from N-epsilon-chloroacetyl-L-lysine. Xaa12 is an amino acid residue derived from L-homocysteine. Xaa2 and Xaa12 are bridged by a thioether bond.
DXAYHWGELVWXTKK

SEQ ID NO: 43 - protein, 15 aa, Artificial Sequence
  Cyclic_peptide_41
  MISC_FEATURE (2)..(2): Xaa2 is an amino acid residue derived from N-epsilon-chloroacetyl-L-lysine. Xaa12 is an amino acid residue derived from L-homocysteine. Xaa2 and Xaa12 are bridged by a thioether bond.
  MISC_FEATURE (12)..(12): Xaa2 is an amino acid residue derived from N-epsilon-chloroacetyl-L-lysine. Xaa12 is an amino acid residue derived from L-homocysteine. Xaa2 and Xaa12 are bridged by a thioether bond.
DXAYHLDELVWXTKK

SEQ ID NO: 44 - protein, 15 aa, Artificial Sequence
  Cyclic_peptide_42
  MISC_FEATURE (2)..(2): Xaa2 is an amino acid residue derived from N-epsilon-chloroacetyl-L-lysine. Xaa12 is an amino acid residue derived from L-homocysteine. Xaa2 and Xaa12 are bridged by a thioether bond.
  MISC_FEATURE (12)..(12): Xaa2 is an amino acid residue derived from N-epsilon-chloroacetyl-L-lysine. Xaa12 is an amino acid residue derived from L-homocysteine. Xaa2 and Xaa12 are bridged by a thioether bond.
DXAYHLEELVWXTKK

SEQ ID NO: 45 - protein, 15 aa, Artificial Sequence
  Cyclic_peptide_43
  MISC_FEATURE (2)..(2): Xaa2 is an amino acid residue derived from N-epsilon-chloroacetyl-L-lysine. Xaa12 is an amino acid residue derived from L-homocysteine. Xaa2 and Xaa12 are bridged by a thioether bond.
  MISC_FEATURE (12)..(12): Xaa2 is an amino acid residue derived from N-epsilon-chloroacetyl-L-lysine. Xaa12 is an amino acid residue derived from L-homocysteine. Xaa2 and Xaa12 are bridged by a thioether bond.
DXAYHLGDLVWXTKK

SEQ ID NO: 46 - protein, 15 aa, Artificial Sequence
  Cyclic_peptide_44
  MISC_FEATURE (2)..(2): Xaa2 is an amino acid residue derived from N-epsilon-chloroacetyl-L-lysine. Xaa12 is an amino acid residue derived from L-homocysteine. Xaa2 and Xaa12 are bridged by a thioether bond.
  MISC_FEATURE (12)..(12): Xaa2 is an amino acid residue derived from N-epsilon-chloroacetyl-L-lysine. Xaa12 is an amino acid residue derived from L-homocysteine. Xaa2 and Xaa12 are bridged by a thioether bond.
DXAYHLGKLVWXTKK

SEQ ID NO: 47 - protein, 15 aa, Artificial Sequence
  Cyclic_peptide_45
  MISC_FEATURE (2)..(2): Xaa2 is an amino acid residue derived from N-epsilon-chloroacetyl-L-lysine. Xaa12 is an amino acid residue derived from L-homocysteine. Xaa2 and Xaa12 are bridged by a thioether bond.
  MISC_FEATURE (12)..(12): Xaa2 is an amino acid residue derived from N-epsilon-chloroacetyl-L-lysine. Xaa12 is an amino acid residue derived from L-homocysteine. Xaa2 and Xaa12 are bridged by a thioether bond.
DXAYHLGRLVWXTKK

SEQ ID NO: 48 - protein, 15 aa, Artificial Sequence
  Cyclic_peptide_46
  MISC_FEATURE (2)..(2): Xaa2 is an amino acid residue derived from N-epsilon-chloroacetyl-L-lysine. Xaa12 is an amino acid residue derived from L-homocysteine. Xaa2 and Xaa12 are bridged by a thioether bond.
  MISC_FEATURE (12)..(12): Xaa2 is an amino acid residue derived from N-epsilon-chloroacetyl-L-lysine. Xaa12 is an amino acid residue derived from L-homocysteine. Xaa2 and Xaa12 are bridged by a thioether bond.
DXAYHLGHLVWXTKK

SEQ ID NO: 49 - protein, 15 aa, Artificial Sequence
  Cyclic_peptide_47
  MISC_FEATURE (2)..(2): Xaa2 is an amino acid residue derived from N-epsilon-chloroacetyl-L-lysine. Xaa12 is an amino acid residue derived from L-homocysteine. Xaa2 and Xaa12 are bridged by a thioether bond.
  MISC_FEATURE (12)..(12): Xaa2 is an amino acid residue derived from N-epsilon-chloroacetyl-L-lysine. Xaa12 is an amino acid residue derived from L-homocysteine. Xaa2 and Xaa12 are bridged by a thioether bond.
DXAYHLGMLVWXTKK

SEQ ID NO: 50 - protein, 15 aa, Artificial Sequence
  Cyclic_peptide_48
  MISC_FEATURE (2)..(2): Xaa2 is an amino acid residue derived from N-epsilon-chloroacetyl-L-lysine. Xaa12 is an amino acid residue derived from L-homocysteine. Xaa2 and Xaa12 are bridged by a thioether bond.
  MISC_FEATURE (12)..(12): Xaa2 is an amino acid residue induced from N-epsilon-chloroacetyl-L-lysine. Xaa12 is an amino acid residue induced from L-homocysteine. Xaa2 and Xaa12 are bridged by a thioether bond.
  MISC_FEATURE (12)..(12): Xaa2 is an amino acid residue derived from N-epsilon-chloroacetyl-L-lysine. Xaa12 is an amino acid residue derived from L-homocysteine. Xaa2 and Xaa12 are bridged by a thioether bond.
DXAYHLGNLVWXTKK

SEQ ID NO: 51 - protein, 15 aa, Artificial Sequence
  Cyclic_peptide_49
  MISC_FEATURE (2)..(2): Xaa2 is an amino acid residue derived from N-epsilon-chloroacetyl-L-lysine. Xaa12 is an amino acid residue derived from L-homocysteine. Xaa2 and Xaa12 are bridged by a thioether bond.
  MISC_FEATURE (12)..(12): Xaa2 is an amino acid residue derived from N-epsilon-chloroacetyl-L-lysine. Xaa12 is an amino acid residue derived from L-homocysteine. Xaa2 and Xaa12 are bridged by a thioether bond.
DXAYHLGEIVWXTKK

SEQ ID NO: 52 - protein, 15 aa, Artificial Sequence
  Cyclic_peptide_50
  MISC_FEATURE (2)..(2): Xaa2 is an amino acid residue derived from N-epsilon-chloroacetyl-L-lysine. Xaa12 is an amino acid residue derived from L-homocysteine. Xaa2 and Xaa12 are bridged by a thioether bond.
  MISC_FEATURE (12)..(12): Xaa2 is an amino acid residue derived from N-epsilon-chloroacetyl-L-lysine. Xaa12 is an amino acid residue derived from L-homocysteine. Xaa2 and Xaa12 are bridged by a thioether bond.
DXAYHLGEMVWXTKK

SEQ ID NO: 53 - protein, 15 aa, Artificial Sequence
  Cyclic_peptide_51
  MISC_FEATURE (2)..(2): Xaa2 is an amino acid residue derived from N-epsilon-chloroacetyl-L-lysine. Xaa12 is an amino acid residue derived from L-homocysteine. Xaa2 and Xaa12 are bridged by a thioether bond.
  MISC_FEATURE (12)..(12): Xaa2 is an amino acid residue derived from N-epsilon-chloroacetyl-L-lysine. Xaa12 is an amino acid residue derived from L-homocysteine. Xaa2 and Xaa12 are bridged by a thioether bond.
DXAYHLGEKVWXTKK

SEQ ID NO: 54 - protein, 15 aa, Artificial Sequence
  Cyclic_peptide_52
  MISC_FEATURE (2)..(2): Xaa2 is an amino acid residue derived from N-epsilon-chloroacetyl-L-lysine. Xaa12 is an amino acid residue derived from L-homocysteine. Xaa2 and Xaa12 are bridged by a thioether bond.
  MISC_FEATURE (12)..(12): Xaa2 is an amino acid residue induced from N-epsilon-chloroacetyl-L-lysine. Xaa12 is an amino acid residue induced from L-homocysteine. Xaa2 and Xaa12 are bridged by a thioether bond.
  MISC_FEATURE (12)..(12): Xaa2 is an amino acid residue derived from N-epsilon-chloroacetyl-L-lysine. Xaa12 is an amino acid residue derived from L-homocysteine. Xaa2 and Xaa12 are bridged by a thioether bond.
DXAYHLGERVWXTKK

SEQ ID NO: 55 - protein, 15 aa, Artificial Sequence
  Cyclic_peptide_53
  MISC_FEATURE (2)..(2): Xaa2 is an amino acid residue derived from N-epsilon-chloroacetyl-L-lysine. Xaa12 is an amino acid residue derived from L-homocysteine. Xaa2 and Xaa12 are bridged by a thioether bond.
  MISC_FEATURE (12)..(12): Xaa2 is an amino acid residue derived from N-epsilon-chloroacetyl-L-lysine. Xaa12 is an amino acid residue derived from L-homocysteine. Xaa2 and Xaa12 are bridged by a thioether bond.
DXAYHLGELIWXTKK

SEQ ID NO: 56 - protein, 15 aa, Artificial Sequence
  Cyclic_peptide_54
  MISC_FEATURE (2)..(2): Xaa2 and Xaa12 are amino acid residues derived from L-homocysteine. Xaa2 and Xaa12 are bridged by a disulfide bond.
  MISC_FEATURE (12)..(12): Xaa2 and Xaa12 are amino acid residues derived from L-homocysteine. Xaa2 and Xaa12 are bridged by a disulfide bond.
DXSYHLGELVWXTKK

SEQ ID NO: 57 - protein, 15 aa, Artificial Sequence
  Cyclic_peptide_55
  MISC_FEATURE (2)..(2): Xaa2 and Xaa12 are amino acid residues derived from L-homocysteine. Xaa2 and Xaa12 are bridged by a disulfide bond.
  MISC_FEATURE (12)..(12): Xaa2 and Xaa12 are amino acid residues derived from L-homocysteine. Xaa2 and Xaa12 are bridged by a disulfide bond..
DXTYHLGELVWXTKK

SEQ ID NO: 58 - protein, 15 aa, Artificial Sequence
  Cyclic_peptide_56
  MISC_FEATURE (2)..(2): Xaa2 and Xaa12 are amino acid residues derived from L-homocysteine. Xaa2 and Xaa12 are bridged by a disulfide bond.
  MISC_FEATURE (12)..(12): Xaa2 and Xaa12 are amino acid residues derived from L-homocysteine. Xaa2 and Xaa12 are bridged by a disulfide bond.
DXAWHLGELVWXTKK

SEQ ID NO: 59 - protein, 15 aa, Artificial Sequence
  Cyclic_peptide_57
  MISC_FEATURE (2)..(2): Xaa2 and Xaa12 are amino acid residues derived from L-homocysteine. Xaa2 and Xaa12 are bridged by a disulfide bond.
  MISC_FEATURE (12)..(12): Xaa2 and Xaa12 are amino acid residues derived from L-homocysteine. Xaa2 and Xaa12 are bridged by a disulfide bond.
DXAFHLGELVWXTKK

SEQ ID NO: 60 - protein, 15 aa, Artificial Sequence
  Cyclic_peptide_58
  MISC_FEATURE (2)..(2): Xaa2 and Xaa12 are amino acid residues derived from L-homocysteine. Xaa2 and Xaa12 are bridged by a disulfide bond.
  MISC_FEATURE (12)..(12): Xaa2 and Xaa12 are amino acid residues derived from L-homocysteine. Xaa2 and Xaa12 are bridged by a disulfide bond.
DXAHHLGELVWXTKK

SEQ ID NO: 61 - protein, 15 aa, Artificial Sequence
  Cyclic_peptide_59
  MISC_FEATURE (2)..(2): Xaa2 and Xaa12 are amino acid residues derived from L-homocysteine. Xaa2 and Xaa12 are bridged by a disulfide bond.
  MISC_FEATURE (12)..(12): Xaa2 and Xaa12 are amino acid residues derived from L-homocysteine. Xaa2 and Xaa12 are bridged by a disulfide bond.
DXAYYLGELVWXTKK

SEQ ID NO: 62 - protein, 15 aa, Artificial Sequence
  Cyclic_peptide_60
  MISC_FEATURE (2)..(2): Xaa2 and Xaa12 are amino acid residues derived from L-homocysteine. Xaa2 and Xaa12 are bridged by a disulfide bond.
  MISC_FEATURE (12)..(12): Xaa2 and Xaa12 are amino acid residues derived from L-homocysteine. Xaa2 and Xaa12 are bridged by a disulfide bond.
DXAYHMGELVWXTKK

SEQ ID NO: 63 - protein, 15 aa, Artificial Sequence
  Cyclic_peptide_61
  MISC_FEATURE (2)..(2): Xaa2 and Xaa12 are amino acid residues derived from L-homocysteine. Xaa2 and Xaa12 are bridged by a disulfide bond.
  MISC_FEATURE (12)..(12): Xaa2 and Xaa12 are amino acid residues derived from L-homocysteine. Xaa2 and Xaa12 are bridged by a disulfide bond.
DXAYHFGELVWXTKK

SEQ ID NO: 64 - protein, 15 aa, Artificial Sequence
  Cyclic_peptide_62
  MISC_FEATURE (2)..(2): Xaa2 and Xaa12 are amino acid residues derived from L-homocysteine. Xaa2 and Xaa12 are bridged by a disulfide bond.
  MISC_FEATURE (12)..(12): Xaa2 and Xaa12 are amino acid residues derived from L-homocysteine. Xaa2 and Xaa12 are bridged by a disulfide bond.
DXAYHHGELVWXTKK

SEQ ID NO: 65 - protein, 15 aa, Artificial Sequence
  Cyclic_peptide_63
  MISC_FEATURE (2)..(2): Xaa2 and Xaa12 are amino acid residues derived from L-homocysteine. Xaa2 and Xaa12 are bridged by a disulfide bond.
  MISC_FEATURE (12)..(12): Xaa2 and Xaa12 are amino acid residues derived from L-homocysteine. Xaa2 and Xaa12 are bridged by a disulfide bond.
DXAYHLGDLVWXTKK

SEQ ID NO: 66 - protein, 15 aa, Artificial Sequence
  Cyclic_peptide_64
  MISC_FEATURE (2)..(2): Xaa2 and Xaa12 are amino acid residues derived from L-homocysteine. Xaa2 and Xaa12 are bridged by a disulfide bond.
  MISC_FEATURE (12)..(12): Xaa2 and Xaa12 are amino acid residues derived from L-homocysteine. Xaa2 and Xaa12 are bridged by a disulfide bond.
DXAYHLGMLVWXTKK

SEQ ID NO: 67 - protein, 15 aa, Artificial Sequence
  Cyclic_peptide_65
  MISC_FEATURE (2)..(2): Xaa2 and Xaa12 are amino acid residues derived from L-homocysteine. Xaa2 and Xaa12 are bridged by a disulfide bond.
  MISC_FEATURE (12)..(12): Xaa2 and Xaa12 are amino acid residues derived from L-homocysteine. Xaa2 and Xaa12 are bridged by a disulfide bond.
DXAYHLGHLVWXTKK

SEQ ID NO: 68 - protein, 15 aa, Artificial Sequence
  Cyclic_peptide_66
  MISC_FEATURE (2)..(2): Xaa2 and Xaa12 are amino acid residues derived from L-homocysteine. Xaa2 and Xaa12 are bridged by a disulfide bond.
  MISC_FEATURE (12)..(12): Xaa2 and Xaa12 are amino acid residues derived from L-homocysteine. Xaa2 and Xaa12 are bridged by a disulfide bond.
DXAYHLGNLVWXTKK

SEQ ID NO: 69 - protein, 15 aa, Artificial Sequence
  Cyclic_peptide_67
  MISC_FEATURE (2)..(2): Xaa2 and Xaa12 are amino acid residues derived from L-homocysteine. Xaa2 and Xaa12 are bridged by a disulfide bond.
  MISC_FEATURE (12)..(12): Xaa2 and Xaa12 are amino acid residues derived from L-homocysteine. Xaa2 and Xaa12 are bridged by a disulfide bond.
DXAYHLGEIVWXTKK

SEQ ID NO: 70 - protein, 15 aa, Artificial Sequence
  Cyclic_peptide_68
  MISC_FEATURE (2)..(2): Xaa2 and Xaa12 are amino acid residues derived from L-homocysteine. Xaa2 and Xaa12 are bridged by a disulfide bond.
  MISC_FEATURE (12)..(12): Xaa2 and Xaa12 are amino acid residues derived from L-homocysteine. Xaa2 and Xaa12 are bridged by a disulfide bond.
DXAYHLGEMVWXTKK

SEQ ID NO: 71 - protein, 15 aa, Artificial Sequence
  Cyclic_peptide_69
  MISC_FEATURE (2)..(2): Xaa2 and Xaa12 are amino acid residues derived from L-homocysteine. Xaa2 and Xaa12 are bridged by a disulfide bond.
  MISC_FEATURE (12)..(12): Xaa2 and Xaa12 are amino acid residues derived from L-homocysteine. Xaa2 and Xaa12 are bridged by a disulfide bond.
DXAYHLGEKVWXTKK

SEQ ID NO: 72 - protein, 15 aa, Artificial Sequence
  Cyclic_peptide_70
  MISC_FEATURE (2)..(2): Xaa2 and Xaa12 are amino acid residues derived from L-homocysteine. Xaa2 and Xaa12 are bridged by a disulfide bond.
  MISC_FEATURE (12)..(12): Xaa2 and Xaa12 are amino acid residues induced from L-homocysteine. Xaa2 and Xaa12 are bridged by a disulfide bond.
  MISC_FEATURE (12)..(12): Xaa2 and Xaa12 are amino acid residues derived from L-homocysteine. Xaa2 and Xaa12 are bridged by a disulfide bond.
DXAYHLGERVWXTKK

SEQ ID NO: 73 - protein, 15 aa, Artificial Sequence
  Cyclic_peptide_71
  MISC_FEATURE (2)..(2): Xaa2 and Xaa12 are amino acid residues derived from L-homocysteine. Xaa2 and Xaa12 are bridged by a disulfide bond.
  MISC_FEATURE (12)..(12): Xaa2 and Xaa12 are amino acid residues derived from L-homocysteine. Xaa2 and Xaa12 are bridged by a disulfide bond.
DXAYHLGELIWXTKK

SEQ ID NO: 74 - protein, 15 aa, Artificial Sequence
  Cyclic_peptide_72
  MISC_FEATURE (2)..(2): Xaa2 is an amino acid residue derived from N-epsilon-chloroacetyl-L-lysine. Xaa12 is an amino acid residue derived from L-penicillamine. Xaa2 and Xaa12 are bridged by a thioether bond.
  MISC_FEATURE (12)..(12): Xaa2 is an amino acid residue derived from N-epsilon-chloroacetyl-L-lysine. Xaa12 is an amino acid residue derived from L-penicillamine. Xaa2 and Xaa12 are bridged by a thioether bond.
DXAYHLGELVWXTKK

SEQ ID NO: 75 - protein, 15 aa, Artificial Sequence
  Cyclic_peptide_73
  MISC_FEATURE (2)..(2): Xaa2 is an amino acid residue derived from L-penicillamine. Xaa12 is an amino acid residue derived from N-epsilon-chloroacetyl-L-lysine. Xaa2 and Xaa12 are bridged by a thioether bond.
  MISC_FEATURE (12)..(12): Xaa2 is an amino acid residue derived from L-penicillamine. Xaa12 is an amino acid residue derived from N-epsilon-chloroacetyl-L-lysine. Xaa2 and Xaa12 are bridged by a thioether bond.
DXAYHLGELVWXTKK

SEQ ID NO: 76 - protein, 15 aa, Artificial Sequence
  Cyclic_peptide_74
  MISC_FEATURE (2)..(2): Xaa2 is an amino acid residue derived from N-epsilon-chloroacetyl-L-lysine. Xaa12 is an amino acid residue derived from L-penicillamine. Xaa2 and Xaa12 are bridged by a thioether bond.
  MISC_FEATURE (12)..(12): Xaa2 is an amino acid residue derived from N-epsilon-chloroacetyl-L-lysine. Xaa12 is an amino acid residue derived from L-penicillamine. Xaa2 and Xaa12 are bridged by a thioether bond.
DXAYHRGELVWXTKK

SEQ ID NO: 77 - protein, 15 aa, Artificial Sequence
  Cyclic_peptide_75
  MISC_FEATURE (2)..(2): Xaa2 is an amino acid residue derived from N-epsilon-chloroacetyl-L-lysine. Xaa12 is an amino acid residue derived from L-penicillamine. Xaa2 and Xaa12 are bridged by a thioether bond.
  MISC_FEATURE (12)..(12): Xaa2 is an amino acid residue derived from N-epsilon-chloroacetyl-L-lysine. Xaa12 is an amino acid residue derived from L-penicillamine. Xaa2 and Xaa12 are bridged by a thioether bond.
  MISC_FEATURE (13)..(13): Xaa13 is an amino acid residue derived from L-homoserine.
DXAYHLGELVWXXKK

SEQ ID NO: 78 - protein, 15 aa, Artificial Sequence
  Cyclic_peptide_76
  MISC_FEATURE (2)..(2): Xaa2 is an amino acid residue derived from (2S)-2-amino-3-[(2-chloroacetyl)amino]propanoic acid. Xaa12 is an amino acid residue derived from L-cysteine. Xaa2 and Xaa12 are bridged by a thioether bond.
  MISC_FEATURE (12)..(12): Xaa2 is an amino acid residue derived from (2S)-2-amino-3-[(2-chloroacetyl)amino]propanoic acid. Xaa12 is an amino acid residue derived from L-cysteine. Xaa2 and Xaa12 are bridged by a thioether bond.
DXAYHLGELVWXTKK

SEQ ID NO: 79 - protein, 15 aa, Artificial Sequence
  Cyclic_peptide_77
  MISC_FEATURE (2)..(2): Xaa2 is an amino acid residue derived from (2S)-2-amino-4-[(2-chloroacetyl)amino]butanoic acid. Xaa12 is an amino acid residue derived from L-cysteine. Xaa2 and Xaa12 are bridged by a thioether bond.
  MISC_FEATURE (12)..(12): Xaa2 is an amino acid residue derived from (2S)-2-amino-4-[(2-chloroacetyl)amino]butanoic acid. Xaa12 is an amino acid residue derived from L-cysteine. Xaa2 and Xaa12 are bridged by a thioether bond.
DXAYHLGELVWXTKK

SEQ ID NO: 80 - protein, 15 aa, Artificial Sequence
  Cyclic_peptide_78
  MISC_FEATURE (2)..(2): Xaa2 is an amino acid residue derived from N-delta-chloroacetyl-L-ornithine. Xaa12 is an amino acid residue derived from L-cysteine. Xaa2 and Xaa12 are bridged by a thioether bond.
  MISC_FEATURE (12)..(12): Xaa2 is an amino acid residue derived from N-delta-chloroacetyl-L-ornithine. Xaa12 is an amino acid residue derived from L-cysteine. Xaa2 and Xaa12 are bridged by a thioether bond.
DXAYHLGELVWXTKK

SEQ ID NO: 81 - protein, 15 aa, Artificial Sequence
  Cyclic_peptide_79
  MISC_FEATURE (2)..(2): Xaa2 is an amino acid residue derived from N-epsilon-chloroacetyl-L-lysine. Xaa12 is an amino acid residue derived from L-cysteine. Xaa2 and Xaa12 are bridged by a thioether bond.
  MISC_FEATURE (12)..(12): Xaa2 is an amino acid residue derived from N-epsilon-chloroacetyl-L-lysine. Xaa12 is an amino acid residue derived from L-cysteine. Xaa2 and Xaa12 are bridged by a thioether bond.
DXAYHLGELVWXTKK

SEQ ID NO: 82 - protein, 15 aa, Artificial Sequence
  Cyclic_peptide_80
  MISC_FEATURE (2)..(2): Xaa2 is an amino acid residue derived from L-cysteine. Xaa12 is an amino acid residue derived from (2S)-2-amino-3-[(2-chloroacetyl)amino]propanoic acid. Xaa2 and Xaa12 are bridged by a thioether bond.
  MISC_FEATURE (12)..(12): Xaa2 is an amino acid residue derived from L-cysteine. Xaa12 is an amino acid residue derived from (2S)-2-amino-3-[(2-chloroacetyl)amino]propanoic acid. Xaa2 and Xaa12 are bridged by a thioether bond.
DXAYHLGELVWXTKK

SEQ ID NO: 83 - protein, 15 aa, Artificial Sequence
  Cyclic_peptide_81
  MISC_FEATURE (2)..(2): Xaa2 is an amino acid residue derived from L-cysteine. Xaa12 is an amino acid residue derived from (2S)-2-amino-4-[(2-chloroacetyl)amino]butanoic acid. Xaa2 and Xaa12 are bridged by a thioether bond.
  MISC_FEATURE (12)..(12): Xaa2 is an amino acid residue derived from L-cysteine. Xaa12 is an amino acid residue derived from (2S)-2-amino-4-[(2-chloroacetyl)amino]butanoic acid. Xaa2 and Xaa12 are bridged by a thioether bond.
DXAYHLGELVWXTKK

SEQ ID NO: 84 - protein, 15 aa, Artificial Sequence
  Cyclic peptide 87
  MISC_FEATURE (2)..(2): Xaa2 is an amino acid residue derived from L-cysteine. Xaa12 is an amino acid residue derived from N-delta-chloroacetyl-L-ornithine. Xaa2 and Xaa12 are bridged by a thioether bond.
  MISC_FEATURE (12)..(12): Xaa2 is an amino acid residue derived from L-cysteine. Xaa12 is an amino acid residue derived from N-delta-chloroacetyl-L-ornithine. Xaa2 and Xaa12 are bridged by a thioether bond.
DXAYHLGELVWXTKK

SEQ ID NO: 85 - protein, 15 aa, Artificial Sequence
  Cyclic_peptide_83
  MISC_FEATURE (2)..(2): Xaa2 is an amino acid residue derived from L-cysteine. Xaa12 is an amino acid residue derived from N-epsilon-chloroacetyl-L-lysine. Xaa2 and Xaa12 are bridged by a thioether bond.
  MISC_FEATURE (12)..(12): Xaa2 is an amino acid residue derived from L-cysteine. Xaa12 is an amino acid residue derived from N-epsilon-chloroacetyl-L-lysine. Xaa2 and Xaa12 are bridged by a thioether bond.
DXAYHLGELVWXTKK

SEQ ID NO: 86 - protein, 15 aa, Artificial Sequence
  Cyclic_peptide_91
  MISC_FEATURE (2)..(2): Xaa2 is an amino acid residue derived from L-glutamic acid. Xaa12 is an amino acid residue derived from L-lysine. Xaa2 and Xaa12 are bridged by an amide bond.
  MISC_FEATURE (12)..(12): Xaa2 is an amino acid residue derived from L-glutamic acid. Xaa12 is an amino acid residue derived from L-lysine. Xaa2 and Xaa12 are bridged by an amide bond.
DXAYHRGELVWXTKK

SEQ ID NO: 87 - protein, 15 aa, Artificial Sequence
  Cyclic_peptide_92
  MISC_FEATURE (2)..(2): Xaa2 and Xaa12 are amino acid residues derived from L-cysteine. Xaa2 and Xaa12 are bridged by a disulfide bond.
  MISC_FEATURE (12)..(12): Xaa2 and Xaa12 are amino acid residues derived from L-cysteine. Xaa2 and Xaa12 are bridged by a disulfide bond.
DXAYHRGELVWXTKK

SEQ ID NO: 88 - protein, 15 aa, Artificial Sequence
  Cyclic_peptide_93
  MISC_FEATURE (2)..(2): Xaa2 is an amino acid residue derived from N-epsilon-chloroacetyl-L-lysine. Xaa12 is an amino acid residue derived from L-penicillamine. Xaa2 and Xaa12 are bridged by a thioether bond.
  MISC_FEATURE (12)..(12): Xaa2 is an amino acid residue derived from N-epsilon-chloroacetyl-L-lysine. Xaa12 is an amino acid residue derived from L-penicillamine. Xaa2 and Xaa12 are bridged by a thioether bond.
DXSYHLGELVWXTKK

SEQ ID NO: 89 - protein, 15 aa, Artificial Sequence
  Cyclic_peptide_94
  MISC_FEATURE (2)..(2): Xaa2 is an amino acid residue derived from N-epsilon-chloroacetyl-L-lysine. Xaa12 is an amino acid residue derived from L-cysteine. Xaa2 and Xaa12 are bridged by a thioether bond.
  MISC_FEATURE (12)..(12): Xaa2 is an amino acid residue derived from N-epsilon-chloroacetyl-L-lysine. Xaa12 is an amino acid residue derived from L-cysteine. Xaa2 and Xaa12 are bridged by a thioether bond.
DXSYHLGELVWXTKK

SEQ ID NO: 90 - protein, 15 aa, Artificial Sequence
  Cyclic_peptide_95
  MISC_FEATURE (2)..(2): Xaa2 is an amino acid residue derived from N-epsilon-chloroacetyl-L-lysine. Xaa12 is an amino acid residue derived from L-cysteine. Xaa2 and Xaa12 are bridged by a thioether bond.
  MISC_FEATURE (12)..(12): Xaa2 is an amino acid residue derived from N-epsilon-chloroacetyl-L-lysine. Xaa12 is an amino acid residue derived from L-cysteine. Xaa2 and Xaa12 are bridged by a thioether bond.
DXAYHRGELVWXTKK

SEQ ID NO: 91 - protein, 15 aa, Artificial Sequence
  Cyclic_peptide_96
  MISC_FEATURE (1)..(1): Xaa1 is an amino acid residue derived from L-homoserine.
  MISC_FEATURE (2)..(2): Xaa2 is an amino acid residue derived from N-epsilon-chloroacetyl-L-lysine. Xaa12 is an amino acid residue derived from L-cysteine. Xaa2 and Xaa12 are bridged by a tioether bond.
  MISC_FEATURE (12)..(12): Xaa2 is an amino acid residue derived from N-epsilon-chloroacetyl-L-lysine. Xaa12 is an amino acid residue derived from L-cysteine. Xaa2 and Xaa12 are bridged by a tioether bond.
XXAYHRGELVWXTKK